European Patent Application EP 4 495 252 A1, published January 22, 2025. Title: 一种对低丰度突变DNA进行富集及检测的方法. Applicant: 广州迪澳基因科技有限公司. Application CN 202210272902.5, filed March 18, 2022. The sequence listing filed with the application follows.

SEQUENCE LISTING (85 sequences)

SEQ ID NO: 1 - DNA, 23 bp, (Artificial Sequence)
  source 1..23: mol_type = other DNA
ggccggtggtcgccgcgatcaag

SEQ ID NO: 2 - DNA, 21 bp, (Artificial Sequence)
  source 1..21: mol_type = other DNA
ccggcacgctcacgtgacaga

SEQ ID NO: 3 - DNA, 27 bp, (Artificial Sequence)
  source 1..27: mol_type = other DNA
cattggcacctgccagctgagccaatg

SEQ ID NO: 4 - DNA, 33 bp, (Artificial Sequence)
  source 1..33: mol_type = other DNA
cctgctcatagaccagaacaacccgctggcagg

SEQ ID NO: 5 - DNA, 31 bp, (Artificial Sequence)
  source 1..31: mol_type = other DNA
cctgctcggggtagacgcacaagcgcgcagg

SEQ ID NO: 6 - DNA, 25 bp, (Artificial Sequence)
  source 1..25: mol_type = other DNA
ctgcccgactgtcggcgctgggcag

SEQ ID NO: 7-10 - skipped (4 entries)

SEQ ID NO: 11 - DNA, 303 bp, (Artificial Sequence)
  source 1..303: mol_type = other DNA
ggagcggatgaccacccaggacgtggaggcgatcacaccgcagacgttgatcaacatccggccggtggtcgccgcgatcaaggagttcttcggcaccagccagctgagccaattcatggaccagaacaacccgctgtcggggttgacccacaagcgccgactgtcggcgctggggcccggcggtctgtcacgtgagcgtgccgggctggaggtccgcgacgtgcacccgtcgcactacggccggatgtgcccgatcgaaacccctgaggggcccaacatcggtctgatcggctcgctgtcggt

SEQ ID NO: 12 - DNA, 303 bp, (Artificial Sequence)
  source 1..303: mol_type = other DNA
ggagcggatgaccacccaggacgtggaggcgatcacaccgcagacgttgatcaacatccggccggtggtcgccgcgatcaaggagttcttcggcaccagccagccgagccaattcatggtccagaacaacccgctgtcggggttgacctacaagcgccgactgttggcgcccgggcccggcggtctgtcacgtgagcgtgccgggctggaggtccgcgacgtgcacccgtcgcactacggccggatgtgcccgatcgaaacccctgaggggcccaacatcggtctgatcggctcgctgtcggt

SEQ ID NO: 13 - DNA, 18 bp, (Artificial Sequence)
  source 1..18: mol_type = other DNA
ggatcctgcgggaagagc

SEQ ID NO: 14 - DNA, 19 bp, (Artificial Sequence)
  source 1..19: mol_type = other DNA
gaaggccatcccggaacag

SEQ ID NO: 15 - DNA, 20 bp, (Artificial Sequence)
  source 1..20: mol_type = other DNA
gcctcatcctggacgtcttc

SEQ ID NO: 16 - DNA, 20 bp, (Artificial Sequence)
  source 1..20: mol_type = other DNA
ggcctcggctgccataaata

SEQ ID NO: 17 - DNA, 23 bp, (Artificial Sequence)
  source 1..23: mol_type = other DNA
cggatacacacatattcatcatc

SEQ ID NO: 18 - DNA, 21 bp, (Artificial Sequence)
  source 1..21: mol_type = other DNA
aatacgccaggcctcacggag

SEQ ID NO: 19-20 - skipped (2 entries)

SEQ ID NO: 21 - DNA, 572 bp, (Artificial Sequence)
  source 1..572: mol_type = other DNA
atggcagagcaggtggccctgagccggacccaggtgtgcgggatcctgcgggaagagcttttccagggcgatgccttccatcagtcggatacacacatattcatcatcatgggtgcatcgggtgacctggccaagaagaagatctaccccaccatctggtggctgttccgggatggccttctgcccgaaaacaccttcatcgtgggctatgcccgttcccgcctcacagtggctgacatccgcaaacagagtgagcccttcttcaaggccaccccagaggagaagctctgatgaccaagaagccgggcatgttcttcaaccccgaggagtcggagctggacctgacctacggcaacagatacaagaacgtgaagctccctgacgcctatgagcgcctcatcctggacgtcttctgcgggagccagatgcacttcgtgcgcagcgacgagctccgtgaggcctggcgtattttcaccccactgctgcaccagattgagctggagaagcccaagcccatcccctatatttatggcagccgaggccccacggaggcagacgagctgatgaagaga

SEQ ID NO: 22 - DNA, 572 bp, (Artificial Sequence)
  source 1..572: mol_type = other DNA
atggcagagcaggtggccctgagccggacccaggtgtgcgggatcctgcgggaagagcttttccagggcgatgccttccatcagtcggatacacgcatattcatcatcatgggtgcatcgggtgacctggccaagaagaagatctaccccaccatctggtggctgttccgggatggccttctgcccgaaaacaccttcatcgtgggctatgcccgttcccgcctcacagtggctgacatccgcaaacagagtgagcccttcttcaaggccaccccagaggagaagctctgatgaccaagaagccgggcatgttcttcaaccccgaggagtcggagctggacctgacctacggcaacagatacaagaacgtgaagctccctgacgcctatgagcgcctcatcctggacgtcttctgcgggagccagatgcacttcgtgcgcagcgacgagctccgtgaggcctggcgtattttcaccccactgctgcaccagattgagctggagaagcccaagcccatcccctatatttatggcagccgaggccccacggaggcagacgagctgatgaagaga

SEQ ID NO: 23 - DNA, 572 bp, (Artificial Sequence)
  source 1..572: mol_type = other DNA
atggcagagcaggtggccctgagccggacccaggtgtgcgggatcctgcgggaagagcttttccagggcgatgccttccatcagtcggatacacacatattcatcatcatgggtgcatcgggtgacctggccaagaagaagatctaccccaccatctggtggctgttccgggatggccttctgcccgaaaacaccttcatcgtgggctatgcccgttcccgcctcacagtggctgacatccgcaaacagagtgagcccttcttcaaggccaccccagaggagaagctctgatgaccaagaagccgggcatgttcttcaaccccgaggagtcggagctggacctgacctacggcaacagatacaagaacgtgaagctccctgacgcctatgagcgcctcatcctggacgtcttctgcgggagccagatgcacttcgtgcgcagcgacgagctccttgaggcctggcgtattttcaccccactgctgcaccagattgagctggagaagcccaagcccatcccctatatttatggcagccgaggccccacggaggcagacgagctgatgaagaga

SEQ ID NO: 24 - DNA, 572 bp, (Artificial Sequence)
  source 1..572: mol_type = other DNA
atggcagagcaggtggccctgagccggacccaggtgtgcgggatcctgcgggaagagcttttccagggcgatgccttccatcagtcggatacacacatattcatcatcatgggtgcatcgggtgacctggccaagaagaagatctaccccaccatctggtggctgttccgggatggccttctgcccgaaaacaccttcatcgtgggctatgcccgttcccgcctcacagtggctgacatccgcaaacagagtgagcccttcttcaaggccaccccagaggagaagctctgatgaccaagaagccgggcatgttcttcaaccccgaggagtcggagctggacctgacctacggcaacagatacaagaacgtgaagctccctgacgcctatgagcgcctcatcctggacgtcttctgcgggagccagatgcacttcgtgcgcagcgacgagctccgtgaggcctggcatattttcaccccactgctgcaccagattgagctggagaagcccaagcccatcccctatatttatggcagccgaggccccacggaggcagacgagctgatgaagaga

SEQ ID NO: 25 - DNA, 22 bp, (Artificial Sequence)
  source 1..22: mol_type = other DNA
actcttcataatgcttgctctg

SEQ ID NO: 26 - DNA, 22 bp, (Artificial Sequence)
  source 1..22: mol_type = other DNA
cctcaattcttaccatccacaa

SEQ ID NO: 27-28 - skipped (2 entries)

SEQ ID NO: 29 - DNA, 493 bp, (Artificial Sequence)
  source 1..493: mol_type = other DNA
tatataggctaaatagaactaatcattgttttagacatacttattgactctaagaggaaagatgaagtactatgttttaaagaatattatattacagaattatagaaattagatctcttacctaaactcttcataatgcttgctctgataggaaaatgagatctactgttttcctttacttactacacctcagatatatttcttcatgaagacctcacagtaaaaataggtgattttggtctagctacagtgaaatctcgatggagtgggtcccatcagtttgaacagttgtctggatccattttgtggatggtaagaattgaggctatttttccactgattaaatttttggccctgagatgctgctgagttactagaaagtcattgaaggtctcaactatagtattttcatagttcccagtattcacaaaaatcagtgttcttattttttatgtccgaaggcagtttgaacagttgtctggatccccttcgg

SEQ ID NO: 30 - DNA, 493 bp, (Artificial Sequence)
  source 1..493: mol_type = other DNA
tatataggctaaatagaactaatcattgttttagacatacttattgactctaagaggaaagatgaagtactatgttttaaagaatattatattacagaattatagaaattagatctcttacctaaactcttcataatgcttgctctgataggaaaatgagatctactgttttcctttacttactacacctcagatatatttcttcatgaagacctcacagtaaaaataggtgattttggtctagctacagagaaatctcgatggagtgggtcccatcagtttgaacagttgtctggatccattttgtggatggtaagaattgaggctatttttccactgattaaatttttggccctgagatgctgctgagttactagaaagtcattgaaggtctcaactatagtattttcatagttcccagtattcacaaaaatcagtgttcttattttttatgtccgaaggcagtttgaacagttgtctggatccccttcgg

SEQ ID NO: 31 - DNA, 20 bp, (Artificial Sequence)
  source 1..20: mol_type = other DNA
atgcaagacaggagccacat

SEQ ID NO: 32 - DNA, 20 bp, (Artificial Sequence)
  source 1..20: mol_type = other DNA
tgggaatgagatagtttctg

SEQ ID NO: 33 - DNA, 20 bp, (Artificial Sequence)
  source 1..20: mol_type = other DNA
agggatccctctgggaagtc

SEQ ID NO: 34 - DNA, 20 bp, (Artificial Sequence)
  source 1..20: mol_type = other DNA
ccacctcggcctcccaaaat

SEQ ID NO: 35 - DNA, 28 bp, (Artificial Sequence)
  source 1..28: mol_type = other DNA
acgaggtccagagataccttgaccttct

SEQ ID NO: 36 - DNA, 26 bp, (Artificial Sequence)
  source 1..26: mol_type = other DNA
acaaccattggccaggtgcggtggct

SEQ ID NO: 37-38 - skipped (2 entries)

SEQ ID NO: 39 - DNA, 133 bp, (Artificial Sequence)
  source 1..133: mol_type = other DNA
atgcaagacaggagccacatgccctacacagatgctgtggtgcacgaggtccagagataccttgaccttctccccaccagcctgccccatgcagtgacctgtgacattaaattcagaaactatctcattccca

SEQ ID NO: 40 - DNA, 133 bp, (Artificial Sequence)
  source 1..133: mol_type = other DNA
atgcaagacaggagccacatgccctacacagatgctgtggtgcacgaggtccagagatacattgaccttctccccaccagcctgccccatgcagtgacctgtgacattaaattcagaaactatctcattccca

SEQ ID NO: 41 - DNA, 105 bp, (Artificial Sequence)
  source 1..105: mol_type = other DNA
agggatccctctgggaagtcaagcaagagaagacctgaaaaacaaccattggccgggtgcggtggctcacgcctataatcctagcattttgggaggccgaggtgg

SEQ ID NO: 42 - DNA, 105 bp, (Artificial Sequence)
  source 1..105: mol_type = other DNA
agggatccctctgggaagtcaagcaagagaagacctgaaaaacaaccattggccaggtgcggtggctcacgcctataatcctagcattttgggaggccgaggtgg

SEQ ID NO: 43 - DNA, 23 bp, (Artificial Sequence)
  source 1..23: mol_type = other DNA
tttsttactgtdgtdgatachac

SEQ ID NO: 44 - DNA, 23 bp, (Artificial Sequence)
  source 1..23: mol_type = other DNA
tttnthachgthgthgayacyac

SEQ ID NO: 45 - DNA, 22 bp, (Artificial Sequence)
  source 1..22: mol_type = other DNA
tttttattacttgtgttgacac

SEQ ID NO: 46 - DNA, 25 bp, (Artificial Sequence)
  source 1..25: mol_type = other DNA
gaaaaayaaaytgtaadtcawaytc

SEQ ID NO: 47 - DNA, 28 bp, (Artificial Sequence)
  source 1..28: mol_type = other DNA
tgtgctgccatatctacttcagaaacta

SEQ ID NO: 48 - DNA, 25 bp, (Artificial Sequence)
  source 1..25: mol_type = other DNA
ttctacacagtctcctgtacctggg

SEQ ID NO: 49 - DNA, 25 bp, (Artificial Sequence)
  source 1..25: mol_type = other DNA
tgcaattgcaaacagtgatactaca

SEQ ID NO: 50 - DNA, 25 bp, (Artificial Sequence)
  source 1..25: mol_type = other DNA
acaagtaactagtgacagtacatat

SEQ ID NO: 51 - DNA, 25 bp, (Artificial Sequence)
  source 1..25: mol_type = other DNA
tgctgtgtctactagtgacagtaca

SEQ ID NO: 52 - DNA, 27 bp, (Artificial Sequence)
  source 1..27: mol_type = other DNA
tctatagagtcttccataccttctaca

SEQ ID NO: 53 - DNA, 26 bp, (Artificial Sequence)
  source 1..26: mol_type = other DNA
tctacacaaaatcctgtgccaaatac

SEQ ID NO: 54 - DNA, 25 bp, (Artificial Sequence)
  source 1..25: mol_type = other DNA
tgccactgctgcggtttccccaaca

SEQ ID NO: 55 - DNA, 25 bp, (Artificial Sequence)
  source 1..25: mol_type = other DNA
tgaggttaaaaaggaaagcacatat

SEQ ID NO: 56 - DNA, 25 bp, (Artificial Sequence)
  source 1..25: mol_type = other DNA
aaccacacagtctatgtctacatat

SEQ ID NO: 57 - DNA, 26 bp, (Artificial Sequence)
  source 1..26: mol_type = other DNA
tgctacagaacagttaagtaaatatg

SEQ ID NO: 58 - DNA, 25 bp, (Artificial Sequence)
  source 1..25: mol_type = other DNA
tgaagtaactaaggaaggtacatat

SEQ ID NO: 59 - DNA, 26 bp, (Artificial Sequence)
  source 1..26: mol_type = other DNA
ttctactacgtcttctattcctaatg

SEQ ID NO: 60 - DNA, 27 bp, (Artificial Sequence)
  source 1..27: mol_type = other DNA
agctaaaagcacattaactaaatatga

SEQ ID NO: 61 - DNA, 25 bp, (Artificial Sequence)
  source 1..25: mol_type = other DNA
tactacagactctactgtaccagct

SEQ ID NO: 62 - DNA, 25 bp, (Artificial Sequence)
  source 1..25: mol_type = other DNA
aggtacacaggctagtagctctact

SEQ ID NO: 63 - DNA, 25 bp, (Artificial Sequence)
  source 1..25: mol_type = other DNA
actgctgctactccatcagttgcac

SEQ ID NO: 64-68 - skipped (5 entries)

SEQ ID NO: 69 - DNA, 142 bp, (Artificial Sequence)
  source 1..142: mol_type = other DNA
tttgttactgttgttgatactacacgcagtacaaatatgtcattatgtgctgccatatctacttcagaaactacatataaaaatactaactttaaggagtacctacgacatggggaggaatatgatttacagtttatttttc

SEQ ID NO: 70 - DNA, 145 bp, (Artificial Sequence)
  source 1..145: mol_type = other DNA
tttgttactgtggtagataccactcccagtaccaatttaacaatatgtgcttctacacagtctcctgtacctgggcaatatgatgctaccaaatttaagcagtatagcagacatgttgaggaatatgatttgcagtttatttttc

SEQ ID NO: 71 - DNA, 142 bp, (Artificial Sequence)
  source 1..142: mol_type = other DNA
tttgttactgtggtagataccacacgcagtaccaatatgtctgtttgtgctgcaattgcaaacagtgatactacatttaaaagtagtaattttaaagagtatttaagacatggtgaggaatttgatttacaatttatatttc

SEQ ID NO: 72 - DNA, 139 bp, (Artificial Sequence)
  source 1..139: mol_type = other DNA
tttgttactgtggtagataccactcgcagtactaatatgactttatgcacacaagtaactagtgacagtacatataaaaatgagaattttaaagaatatataagacatgttgaagaatatgatctacagtttgtttttc

SEQ ID NO: 73 - DNA, 142 bp, (Artificial Sequence)
  source 1..142: mol_type = other DNA
tttgttactgtagttgatacaacccgtagtacaaatatgtctgtgtgttctgctgtgtctactagtgacagtacatataaaaatgacaattttaaggaatatttaaggcatggtgaagaatatgatttacagtttatttttc

SEQ ID NO: 74 - DNA, 145 bp, (Artificial Sequence)
  source 1..145: mol_type = other DNA
tttcttactgtagtggacactacccgtagtaccaactttacattatctacctctatagagtcttccataccttctacatatgatccttctaagtttaaggaatataccaggcacgtggaggagtatgatttacaatttatatttc

SEQ ID NO: 75 - DNA, 145 bp, (Artificial Sequence)
  source 1..145: mol_type = other DNA
tttgttactgtagtggacactacccgcagtactaatttaacattatgtgcctctacacaaaatcctgtgccaaatacatatgatcctactaagtttaagcactatagtagacatgtggaggaatatgatttacagtttatttttc

SEQ ID NO: 76 - DNA, 142 bp, (Artificial Sequence)
  source 1..142: mol_type = other DNA
tttattacctgtgttgatactaccagaagtacaaatttaactattagcactgccactgctgcggtttccccaacatttactccaagtaactttaagcaatatattaggcatggggaagagtatgaattgcaatttatttttc

SEQ ID NO: 77 - DNA, 139 bp, (Artificial Sequence)
  source 1..139: mol_type = other DNA
tttgtcacagttgtggataccactcgtagcactaacatgactttatgtgctgaggttaaaaaggaaagcacatataaaaatgaaaattttaaggaataccttcgtcatggcgaggaatttgatttacaatttatttttc

SEQ ID NO: 78 - DNA, 139 bp, (Artificial Sequence)
  source 1..139: mol_type = other DNA
tttgtaactgttgtggataccaccaggaatacaaacatgactctttccgcaaccacacagtctatgtctacatataattcaaagcaaattaaacagtatgttagacatgcagaggaatatgaattacaatttgtgtttc

SEQ ID NO: 79 - DNA, 139 bp, (Artificial Sequence)
  source 1..139: mol_type = other DNA
tttgttactgtagtagatactactagaagtactaacatgactattagtactgctacagaacagttaagtaaatatgatgcacgaaaaattaatcagtaccttagacatgtggaggaatatgaattacaatttgtttttc

SEQ ID NO: 80 - DNA, 139 bp, (Artificial Sequence)
  source 1..139: mol_type = other DNA
tttgttaccgtcgttgataccactcgtagcactaatatgacattatgcactgaagtaactaaggaaggtacatataaaaatgataattttaaggaatatgtacgtcatgttgaagaatatgacttacagtttgtttttc

SEQ ID NO: 81 - DNA, 145 bp, (Artificial Sequence)
  source 1..145: mol_type = other DNA
tttttaacagttgtagatactactcgcagcaccaatctttctgtgtgtgcttctactacgtcttctattcctaatgtatacacacctaccagttttaaagaatatgccagacatgtggaggaatttgatttgcagtttatatttc

SEQ ID NO: 82 - DNA, 139 bp, (Artificial Sequence)
  source 1..139: mol_type = other DNA
tttgttactgttgtggatactaccagaagcaccaacatgactattaatgcagctaaaagcacattaactaaatatgatgcccgtgaaatcaatcaataccttcgccatgtggaggaatatgaactacagtttgtgtttc

SEQ ID NO: 83 - DNA, 145 bp, (Artificial Sequence)
  source 1..145: mol_type = other DNA
tttcttaccgttgtggatacaacgcgcagtactaattttacattgtccactactacagactctactgtaccagctgtttatgattctaataaatttaaggaatatgttaggcatgttgaggaatatgatttgcagtttatatttc

SEQ ID NO: 84 - DNA, 148 bp, (Artificial Sequence)
  source 1..148: mol_type = other DNA
tttttaactgttgtagatactactagaagcactaatttttctgtatgtgtaggtacacaggctagtagctctactacaacgtatgccaactctaattttaaagaatatttaagacatgcagaagagtatgatttacagtttgtttttc

SEQ ID NO: 85 - DNA, 147 bp, (Artificial Sequence)
  source 1..147: mol_type = other DNA
tttttattacttgtgttgacactaccagaagtactaatttaaccattagcactgctgctactccatcagttgcacagacattcactccaacaaactttaagcagtatattaggcacggggaagaatatgaattacaatttatttttc